European Patent Specification EP 4 036 119 B1, published July 2, 2025. Title: Antibodies Against Claudin 18.2 Useful In Cancer Diagnosis. Applicant: Astellas Pharma Inc., et al. The sequence listing filed with the application follows.

SEQUENCE LISTING (25 sequences)

SEQ ID NO: 1 - protein, 261 aa, Homo sapiens
MSTTTCQVVAFLLSILGLAGCIAATGMDMWSTQDLYDNPVTSVFQYEGLWRSCVRQSSGFTECRPYFTILGLPAMLQAVRALMIVGIVLGAIGLLVSIFALKCIRIGSMEDSAKANMTLTSGIMFIVSGLCAIAGVSVFANMLVTNFWMSTANMYTGMGGMVQTVQTRYTFGAALFVGWVAGGLTLIGGVMMCIACRGLAPEETNYKAVSYHASGHSVAYKPGGFKASTGFGSNTKNKKIYDGGARTEDEVQSYPSKHDYV

SEQ ID NO: 2 - protein, 261 aa, Homo sapiens
MAVTACQGLGFVVSLIGIAGIIAATCMDQWSTQDLYNNPVTAVFNYQGLWRSCVRESSGFTECRGYFTLLGLPAMLQAVRALMIVGIVLGAIGLLVSIFALKCIRIGSMEDSAKANMTLTSGIMFIVSGLCAIAGVSVFANMLVTNFWMSTANMYTGMGGMVQTVQTRYTFGAALFVGWVAGGLTLIGGVMMCIACRGLAPEETNYKAVSYHASGHSVAYKPGGFKASTGFGSNTKNKKIYDGGARTEDEVQSYPSKHDYV

SEQ ID NO: 3 - protein, 264 aa, Mus musculus
MSVTACQGLGFVVSLIGFAGIIAATCMDQWSTQDLYNNPVTAVFNYQGLWRSCVRESSGFTECRGYFTLLGLPAMLQAVRALMIVGIVLGVIGILVSIFALKCIRIGSMDDSAKAKMTLTSGILFIISGICAIIGVSVFANMLVTNFWMSTANMYSGMGGMGGMVQTVQTRYTFGAALFVGWVAGGLTLIGGVMMCIACRGLTPDDSNFKAVSYHASGQNVAYRPGGFKASTGFGSNTRNKKIYDGGARTEDDEQSHPTKYDYV

SEQ ID NO: 4 - protein, 261 aa, Artificial Sequence
  Consensus Sequence
  MISC_FEATURE (18)..(18): Variable Amino Acid
MSVTACQGLGFVVSLIGXAGIIAATCMDQWSTQDLYNNPVTAVFNYQGLWRSCVRESSGFTECRGYFTLLGLPAMLQAVRALMIVGIVLGAIGLLVSIFALKCIRIGSMEDSAKANMTLTSGIMFIVSGLCAIAGVSVFANMLVTNFWMSTANMYTGMGGMVQTVQTRYTFGAALFVGWVAGGLTLIGGVMMCIACRGLAPEETNYKAVSYHASGHSVAYKPGGFKASTGFGSNTKNKKIYDGGARTEDEVQSYPSKHDYV

SEQ ID NO: 5 - protein, 15 aa, Artificial Sequence
  Peptide For Immunization
TEDEVQSYPSKHDYV

SEQ ID NO: 6 - protein, 12 aa, Artificial Sequence
  Peptide For Immunization
EVQSYPSKHDYV

SEQ ID NO: 7 - protein, 134 aa, Mus musculus
MAWVWTLLFLMAAAQSIQAQIQLVQSGPELKKFGETVKISCKASGYTFTDYSIHWVKQAPGKGLKWMGWINTETGVPTYADDFKGRFAFSLETSASTAYLQINNLKNEDTATYFCARRTGFDYWGQGTTLTVSS

SEQ ID NO: 8 - protein, 8 aa, Mus musculus
GYTFTDYS

SEQ ID NO: 9 - protein, 8 aa, Mus musculus
INTETGVP

SEQ ID NO: 10 - protein, 8 aa, Mus musculus
ARRTGFDY

SEQ ID NO: 11 - protein, 132 aa, Mus musculus
MRFSAQLLGLLVLWIPGSTADIVMTQAAFSIPVTLGTSASISCRSSKNLLHSDGITYLYWYLQRPGQSPQLLIYRVSNLASGVPNRFSGSESGTDFTLRISRVEAEDVGVYYCVQVLELPFTFGGGTKLEIK

SEQ ID NO: 12 - protein, 11 aa, Mus musculus
KNLLHSDGITY

SEQ ID NO: 13 - protein, 3 aa, Mus musculus
RVS

SEQ ID NO: 14 - protein, 9 aa, Mus musculus
VQVLELPFT

SEQ ID NO: 15 - protein, 140 aa, Mus musculus
MNFGLSLIFLVLVLKGVQCEVHLVESGGGLVKPGGSLKLSCAASGFTFSSYAMSWVRQTPEKRLEWVATISDGGSYSYYPDNVKGRFTISRDNAKNNLYLQMSHLKSEDTAIYYCARDSYYDNSYVRDYWGQGTTLTVSS

SEQ ID NO: 16 - protein, 8 aa, Mus musculus
GFTFSSYA

SEQ ID NO: 17 - protein, 8 aa, Mus musculus
ISDGGSYS

SEQ ID NO: 18 - protein, 14 aa, Mus musculus
ARDSYYDNSYVRDY

SEQ ID NO: 19 - protein, 127 aa, Mus musculus
MRTPAQFLGILLLWFPGIKCDIKMTQSPSSMYASLGERVSITCKASQDINTFLSWFQQKPGKSPKTLIYRTNRLIDGVPSRFSGSGSGQDYSLTISSLDYEDMGIYYCLQYDEFPLTFGAGTKLELK

SEQ ID NO: 20 - protein, 6 aa, Mus musculus
QDINTF

SEQ ID NO: 21 - protein, 3 aa, Mus musculus
RTN

SEQ ID NO: 22 - protein, 9 aa, Mus musculus
LQYDEFPLT

SEQ ID NO: 23 - DNA, 330 bp, Artificial Sequence
  Nucleic Acid Encoding Peptide For Immunization
atgcggggttctcatcatcatcatcatcatggtatggctagcatgactggtggacagcaaatgggtcgggatctgtacgacgatgacgataaggatcgatggggatccgagctcgagatgatgtgcatcgcctgccggggcctggcaccagaagaaaccaactacaaagccgtttcttatcatgcctcgggccacagtgttgcctacaagcctggaggcttcaaggccagcactggctttgggtccaacaccaaaaacaagaagatatacgatggaggtgcccgcacagaggacgaggtacaatcttatccttccaagcacgactatgtg

SEQ ID NO: 24 - protein, 110 aa, Artificial Sequence [sequence omitted]

SEQ ID NO: 25 - protein, 71 aa, Artificial Sequence
  Peptide For Immunization
MMCIACRGLAPEETNYKAVSYHASGHSVAYKPGGFKASTGFGSNTKNKKIYDGGARTEDEVQSYPSKHDYV